European Patent Application EP 4 289 971 A1, published December 13, 2023. Title: Methylation-specific primers for diagnosing tumors. Applicant: Heinrich-Heine-Universität Düsseldorf. The sequence listing filed with the application follows.

SEQUENCE LISTING (182 sequences)

SEQ ID NO: 1 - DNA, 1100 bp, Homo sapiens
gggaagtcctcagctgtcctgcggttgtgccggggccccaggtctggaggggaccagtggccgtgtggcttctactgctgggctggaagtcgggcctcctagctctgcagtccgaggcttggagccaggtgcctggaccccgaggctgccctccaccctgtgcgggcgggatgtgaccagatgttggcctcatctgccagacagagtgccggggcccagggtcaaggccgttgtggctggtgtgaggcgcccggtgcgcggccagcaggagcgcctggctccatttcccaccctttctcgacgggaccgccccggtgggtgattaacagatttggggtggtttgctcatggtggggacccctcgccgcctgagaacctgcaaagagaaatgacgggcctgtgtcaaggagcccaagtcgcggggaagtgttgcagggaggcactccgggaggtcccgcgtgcccgtccagggagcaatgcgtcctcgggttcgtccccagccgcgtctacgcgcctccgtcctccccttcacgtccggcattcgtggtgcccggagcccgacgccccgcgtccggacctggaggcagccctgggtctccggatcaggccagcggccaaagggtcgccgcacgcacctgttcccagggcctccacatcatggcccctccctcgggttaccccacagcctaggccgattcgacctctctccgctggggccctcgctggcgtccctgcaccctgggagcgcgagcggcgcgcgggcggggaagcgcggcccagacccccgggtccgcccggagcagctgcgctgtcggggccaggccgggctcccagtggattcgcgggcacagacgcccaggaccgcgctccccacgtggcggagggactggggacccgggcacccgtcctgccccttcaccttccagctccgcctcctccgcgcggaccccgccccgtcccgacccctcccgggtccccggcccagccccctccgggccctcccagcccctccccttcctttccgcggccccgccctctcctcgcggcgcgagtttcaggcagcgctgcgtcctgctgcgcacgtgggaagccctggcccc

SEQ ID NO: 2 - DNA, 1100 bp, Artificial sequence
  Bisulfite converted, amplified sequence of SEQ ID NO:1 in a case where all of the CpG dinucleotides were methylated
gggaagtttttagttgttttgcggttgtgtcggggttttaggtttggaggggattagtggtcgtgtggtttttattgttgggttggaagtcgggttttttagttttgtagttcgaggtttggagttaggtgtttggatttcgaggttgttttttattttgtgcgggcgggatgtgattagatgttggttttatttgttagatagagtgtcggggtttagggttaaggtcgttgtggttggtgtgaggcgttcggtgcgcggttagtaggagcgtttggttttattttttattttttttcgacgggatcgtttcggtgggtgattaatagatttggggtggtttgtttatggtggggatttttcgtcgtttgagaatttgtaaagagaaatgacgggtttgtgttaaggagtttaagtcgcggggaagtgttgtagggaggtatttcgggaggtttcgcgtgttcgtttagggagtaatgcgttttcgggttcgtttttagtcgcgtttacgcgttttcgtttttttttttacgttcggtattcgtggtgttcggagttcgacgtttcgcgttcggatttggaggtagttttgggttttcggattaggttagcggttaaagggtcgtcgtacgtatttgtttttagggtttttatattatggtttttttttcgggttattttatagtttaggtcgattcgattttttttcgttggggttttcgttggcgtttttgtattttgggagcgcgagcggcgcgcgggcggggaagcgcggtttagattttcgggttcgttcggagtagttgcgttgtcggggttaggtcgggtttttagtggattcgcgggtatagacgtttaggatcgcgttttttacgtggcggagggattggggattcgggtattcgttttgtttttttattttttagtttcgtttttttcgcgcggattttgtttcgtttcgatttttttcgggttttcggtttagtttttttcgggtttttttagtttttttttttttttttcgcggtttcgtttttttttcgcggcgcgagttttaggtagcgttgcgttttgttgcgtacgtgggaagttttggtttt

SEQ ID NO: 3 - DNA, 1100 bp, Artificial sequence
  Reverse complement of SEQ ID NO: 2
aaaaccaaaacttcccacgtacgcaacaaaacgcaacgctacctaaaactcgcgccgcgaaaaaaaaacgaaaccgcgaaaaaaaaaaaaaaaaactaaaaaaacccgaaaaaaactaaaccgaaaacccgaaaaaaatcgaaacgaaacaaaatccgcgcgaaaaaaacgaaactaaaaaataaaaaaacaaaacgaatacccgaatccccaatccctccgccacgtaaaaaacgcgatcctaaacgtctatacccgcgaatccactaaaaacccgacctaaccccgacaacgcaactactccgaacgaacccgaaaatctaaaccgcgcttccccgcccgcgcgccgctcgcgctcccaaaatacaaaaacgccaacgaaaaccccaacgaaaaaaaatcgaatcgacctaaactataaaataacccgaaaaaaaaaccataatataaaaaccctaaaaacaaatacgtacgacgaccctttaaccgctaacctaatccgaaaacccaaaactacctccaaatccgaacgcgaaacgtcgaactccgaacaccacgaataccgaacgtaaaaaaaaaaacgaaaacgcgtaaacgcgactaaaaacgaacccgaaaacgcattactccctaaacgaacacgcgaaacctcccgaaatacctccctacaacacttccccgcgacttaaactccttaacacaaacccgtcatttctctttacaaattctcaaacgacgaaaaatccccaccataaacaaaccaccccaaatctattaatcacccaccgaaacgatcccgtcgaaaaaaaataaaaaataaaaccaaacgctcctactaaccgcgcaccgaacgcctcacaccaaccacaacgaccttaaccctaaaccccgacactctatctaacaaataaaaccaacatctaatcacatcccgcccgcacaaaataaaaaacaacctcgaaatccaaacacctaactccaaacctcgaactacaaaactaaaaaacccgacttccaacccaacaataaaaaccacacgaccactaatcccctccaaacctaaaaccccgacacaaccgcaaaacaactaaaaacttccc

SEQ ID NO: 4 - DNA, 1100 bp, Artificial sequence
  Bisulfite converted, amplified sequence of SEQ ID NO:1 in a case where all of the CpG dinucleotides were unmethylated
gggaagtttttagttgttttgtggttgtgttggggttttaggtttggaggggattagtggttgtgtggtttttattgttgggttggaagttgggttttttagttttgtagtttgaggtttggagttaggtgtttggattttgaggttgttttttattttgtgtgggtgggatgtgattagatgttggttttatttgttagatagagtgttggggtttagggttaaggttgttgtggttggtgtgaggtgtttggtgtgtggttagtaggagtgtttggttttattttttatttttttttgatgggattgttttggtgggtgattaatagatttggggtggtttgtttatggtggggattttttgttgtttgagaatttgtaaagagaaatgatgggtttgtgttaaggagtttaagttgtggggaagtgttgtagggaggtattttgggaggttttgtgtgtttgtttagggagtaatgtgtttttgggtttgtttttagttgtgtttatgtgtttttgtttttttttttatgtttggtatttgtggtgtttggagtttgatgttttgtgtttggatttggaggtagttttgggtttttggattaggttagtggttaaagggttgttgtatgtatttgtttttagggtttttatattatggttttttttttgggttattttatagtttaggttgatttgatttttttttgttggggtttttgttggtgtttttgtattttgggagtgtgagtggtgtgtgggtggggaagtgtggtttagatttttgggtttgtttggagtagttgtgttgttggggttaggttgggtttttagtggatttgtgggtatagatgtttaggattgtgttttttatgtggtggagggattggggatttgggtatttgttttgtttttttattttttagttttgttttttttgtgtggattttgttttgttttgattttttttgggtttttggtttagttttttttgggtttttttagttttttttttttttttttgtggttttgttttttttttgtggtgtgagttttaggtagtgttgtgttttgttgtgtatgtgggaagttttggtttt

SEQ ID NO: 5 - DNA, 1100 bp, Artificial sequence
  Reverse complement of SEQ ID NO: 4
aaaaccaaaacttcccacatacacaacaaaacacaacactacctaaaactcacaccacaaaaaaaaaacaaaaccacaaaaaaaaaaaaaaaaaactaaaaaaacccaaaaaaaactaaaccaaaaacccaaaaaaaatcaaaacaaaacaaaatccacacaaaaaaaacaaaactaaaaaataaaaaaacaaaacaaatacccaaatccccaatccctccaccacataaaaaacacaatcctaaacatctatacccacaaatccactaaaaacccaacctaaccccaacaacacaactactccaaacaaacccaaaaatctaaaccacacttccccacccacacaccactcacactcccaaaatacaaaaacaccaacaaaaaccccaacaaaaaaaaatcaaatcaacctaaactataaaataacccaaaaaaaaaaccataatataaaaaccctaaaaacaaatacatacaacaaccctttaaccactaacctaatccaaaaacccaaaactacctccaaatccaaacacaaaacatcaaactccaaacaccacaaataccaaacataaaaaaaaaaacaaaaacacataaacacaactaaaaacaaacccaaaaacacattactccctaaacaaacacacaaaacctcccaaaatacctccctacaacacttccccacaacttaaactccttaacacaaacccatcatttctctttacaaattctcaaacaacaaaaaatccccaccataaacaaaccaccccaaatctattaatcacccaccaaaacaatcccatcaaaaaaaaataaaaaataaaaccaaacactcctactaaccacacaccaaacacctcacaccaaccacaacaaccttaaccctaaaccccaacactctatctaacaaataaaaccaacatctaatcacatcccacccacacaaaataaaaaacaacctcaaaatccaaacacctaactccaaacctcaaactacaaaactaaaaaacccaacttccaacccaacaataaaaaccacacaaccactaatcccctccaaacctaaaaccccaacacaaccacaaaacaactaaaaacttccc

SEQ ID NO: 6 - DNA, 269 bp, Homo sapiens
gggcctgtgtcaaggagcccaagtcgcggggaagtgttgcagggaggcactccgggaggtcccgcgtgcccgtccagggagcaatgcgtcctcgggttcgtccccagccgcgtctacgcgcctccgtcctccccttcacgtccggcattcgtggtgcccggagcccgacgccccgcgtccggacctggaggcagccctgggtctccggatcaggccagcggccaaagggtcgccgcacgcacctgttcccagggcctccacatcatggc

SEQ ID NO: 7 - DNA, 269 bp, Artificial sequence
  Bisulfite converted, amplified sequence of SEQ ID NO:6 in a case where all of the CpG dinucleotides were methylated
gggtttgtgttaaggagtttaagtcgcggggaagtgttgtagggaggtatttcgggaggtttcgcgtgttcgtttagggagtaatgcgttttcgggttcgtttttagtcgcgtttacgcgttttcgtttttttttttacgttcggtattcgtggtgttcggagttcgacgtttcgcgttcggatttggaggtagttttgggttttcggattaggttagcggttaaagggtcgtcgtacgtatttgtttttagggtttttatattatggt

SEQ ID NO: 8 - DNA, 269 bp, Artificial sequence
  Reverse complement of SEQ ID NO: 7
accataatataaaaaccctaaaaacaaatacgtacgacgaccctttaaccgctaacctaatccgaaaacccaaaactacctccaaatccgaacgcgaaacgtcgaactccgaacaccacgaataccgaacgtaaaaaaaaaaacgaaaacgcgtaaacgcgactaaaaacgaacccgaaaacgcattactccctaaacgaacacgcgaaacctcccgaaatacctccctacaacacttccccgcgacttaaactccttaacacaaaccc

SEQ ID NO: 9 - DNA, 269 bp, Artificial sequence
  Bisulfite converted, amplified sequence of SEQ ID NO:6 in a case where all of the CpG dinucleotides were unmethylated
gggtttgtgttaaggagtttaagttgtggggaagtgttgtagggaggtattttgggaggttttgtgtgtttgtttagggagtaatgtgtttttgggtttgtttttagttgtgtttatgtgtttttgtttttttttttatgtttggtatttgtggtgtttggagtttgatgttttgtgtttggatttggaggtagttttgggtttttggattaggttagtggttaaagggttgttgtatgtatttgtttttagggtttttatattatggt

SEQ ID NO: 10 - DNA, 269 bp, Artificial sequence
  Reverse complement of SEQ ID NO: 10
accataatataaaaaccctaaaaacaaatacatacaacaaccctttaaccactaacctaatccaaaaacccaaaactacctccaaatccaaacacaaaacatcaaactccaaacaccacaaataccaaacataaaaaaaaaaacaaaaacacataaacacaactaaaaacaaacccaaaaacacattactccctaaacaaacacacaaaacctcccaaaatacctccctacaacacttccccacaacttaaactccttaacacaaaccc

SEQ ID NO: 11 - DNA, 25 bp, Artificial sequence
  An exemplary methylation-specific primer (sense)
tttttagttgttttgcggttgtgtc

SEQ ID NO: 12 - DNA, 25 bp, Artificial sequence
  An exemplary methylation-specific primer (sense)
ttcgaggttgttttttattttgtgc

SEQ ID NO: 13 - DNA, 25 bp, Artificial sequence
  An exemplary methylation-specific primer (sense)
aggttgttttttattttgtgcgggc

SEQ ID NO: 14 - DNA, 25 bp, Artificial sequence
  An exemplary methylation-specific primer (sense)
agtgtcggggtttagggttaaggtc

SEQ ID NO: 15 - DNA, 25 bp, Artificial sequence
  An exemplary methylation-specific primer (sense)
aaggtcgttgtggttggtgtgaggc

SEQ ID NO: 16 - DNA, 25 bp, Artificial sequence
  An exemplary methylation-specific primer (sense)
tcgttgtggttggtgtgaggcgttc

SEQ ID NO: 17 - DNA, 25 bp, Artificial sequence
  An exemplary methylation-specific primer (sense)
gtggttggtgtgaggcgttcggtgc

SEQ ID NO: 18 - DNA, 25 bp, Artificial sequence
  An exemplary methylation-specific primer (sense)
ggttggtgtgaggcgttcggtgcgc

SEQ ID NO: 19 - DNA, 25 bp, Artificial sequence
  An exemplary methylation-specific primer (sense)
cgttcggtgcgcggttagtaggagc

SEQ ID NO: 20 - DNA, 25 bp, Artificial sequence
  An exemplary methylation-specific primer (sense)
ttggttttattttttattttttttc

SEQ ID NO: 21 - DNA, 25 bp, Artificial sequence
  An exemplary methylation-specific primer (sense)
gttttattttttattttttttcgac

SEQ ID NO: 22 - DNA, 25 bp, Artificial sequence
  An exemplary methylation-specific primer (sense)
ttttttattttttttcgacgggatc

SEQ ID NO: 23 - DNA, 25 bp, Artificial sequence
  An exemplary methylation-specific primer (sense)
tattttttttcgacgggatcgtttc

SEQ ID NO: 24 - DNA, 25 bp, Artificial sequence
  An exemplary methylation-specific primer (sense)
ttgtttatggtggggatttttcgtc

SEQ ID NO: 25 - DNA, 25 bp, Artificial sequence
  An exemplary methylation-specific primer (sense)
gggtttgtgttaaggagtttaagtc

SEQ ID NO: 26 - DNA, 25 bp, Artificial sequence
  An exemplary methylation-specific primer (sense)
gtttgtgttaaggagtttaagtcgc

SEQ ID NO: 27 - DNA, 25 bp, Artificial sequence
  An exemplary methylation-specific primer (sense)
gtagggaggtatttcgggaggtttc

SEQ ID NO: 28 - DNA, 25 bp, Artificial sequence
  An exemplary methylation-specific primer (sense)
agggaggtatttcgggaggtttcgc

SEQ ID NO: 29 - DNA, 25 bp, Artificial sequence
  An exemplary methylation-specific primer (sense)
gtatttcgggaggtttcgcgtgttc

SEQ ID NO: 30 - DNA, 25 bp, Artificial sequence
  An exemplary methylation-specific primer (sense)
cgcgtgttcgtttagggagtaatgc

SEQ ID NO: 31 - DNA, 25 bp, Artificial sequence
  An exemplary methylation-specific primer (sense)
ttcgtttagggagtaatgcgttttc

SEQ ID NO: 32 - DNA, 25 bp, Artificial sequence
  An exemplary methylation-specific primer (sense)
tagggagtaatgcgttttcgggttc

SEQ ID NO: 33 - DNA, 25 bp, Artificial sequence
  An exemplary methylation-specific primer (sense)
tgcgttttcgggttcgtttttagtc

SEQ ID NO: 34 - DNA, 25 bp, Artificial sequence
  An exemplary methylation-specific primer (sense)
cgttttcgggttcgtttttagtcgc

SEQ ID NO: 35 - DNA, 25 bp, Artificial sequence
  An exemplary methylation-specific primer (sense)
cgggttcgtttttagtcgcgtttac

SEQ ID NO: 36 - DNA, 25 bp, Artificial sequence
  An exemplary methylation-specific primer (sense)
ggttcgtttttagtcgcgtttacgc

SEQ ID NO: 37 - DNA, 25 bp, Artificial sequence
  An exemplary methylation-specific primer (sense)
tttttagtcgcgtttacgcgttttc

SEQ ID NO: 38 - DNA, 25 bp, Artificial sequence
  An exemplary methylation-specific primer (sense)
tacgcgttttcgtttttttttttac

SEQ ID NO: 39 - DNA, 25 bp, Artificial sequence
  An exemplary methylation-specific primer (sense)
cgttttcgtttttttttttacgttc

SEQ ID NO: 40 - DNA, 25 bp, Artificial sequence
  An exemplary methylation-specific primer (sense)
gtttttttttttacgttcggtattc

SEQ ID NO: 41 - DNA, 25 bp, Artificial sequence
  An exemplary methylation-specific primer (sense)
tttacgttcggtattcgtggtgttc

SEQ ID NO: 42 - DNA, 25 bp, Artificial sequence
  An exemplary methylation-specific primer (sense)
tcggtattcgtggtgttcggagttc

SEQ ID NO: 43 - DNA, 25 bp, Artificial sequence
  An exemplary methylation-specific primer (sense)
gtattcgtggtgttcggagttcgac

SEQ ID NO: 44 - DNA, 25 bp, Artificial sequence
  An exemplary methylation-specific primer (sense)
cgtggtgttcggagttcgacgtttc

SEQ ID NO: 45 - DNA, 25 bp, Artificial sequence
  An exemplary methylation-specific primer (sense)
tggtgttcggagttcgacgtttcgc

SEQ ID NO: 46 - DNA, 25 bp, Artificial sequence
  An exemplary methylation-specific primer (sense)
gttcggagttcgacgtttcgcgttc

SEQ ID NO: 47 - DNA, 25 bp, Artificial sequence
  An exemplary methylation-specific primer (sense)
ttttgggttttcggattaggttagc

SEQ ID NO: 48 - DNA, 25 bp, Artificial sequence
  An exemplary methylation-specific primer (sense)
ggattaggttagcggttaaagggtc

SEQ ID NO: 49 - DNA, 25 bp, Artificial sequence
  An exemplary methylation-specific primer (sense)
ttaggttagcggttaaagggtcgtc

SEQ ID NO: 50 - DNA, 25 bp, Artificial sequence
  An exemplary methylation-specific primer (sense)
gttagcggttaaagggtcgtcgtac

SEQ ID NO: 51 - DNA, 25 bp, Artificial sequence
  An exemplary methylation-specific primer (sense)
ttcgggttattttatagtttaggtc

SEQ ID NO: 52 - DNA, 25 bp, Artificial sequence
  An exemplary methylation-specific primer (sense)
gttattttatagtttaggtcgattc

SEQ ID NO: 53 - DNA, 25 bp, Artificial sequence
  An exemplary methylation-specific primer (sense)
gtttaggtcgattcgattttttttc

SEQ ID NO: 54 - DNA, 25 bp, Artificial sequence
  An exemplary methylation-specific primer (sense)
tcgattttttttcgttggggttttc

SEQ ID NO: 55 - DNA, 25 bp, Artificial sequence
  An exemplary methylation-specific primer (sense)
ttttttcgttggggttttcgttggc

SEQ ID NO: 56 - DNA, 25 bp, Artificial sequence
  An exemplary methylation-specific primer (sense)
gttggcgtttttgtattttgggagc

SEQ ID NO: 57 - DNA, 25 bp, Artificial sequence
  An exemplary methylation-specific primer (sense)
tggcgtttttgtattttgggagcgc

SEQ ID NO: 58 - DNA, 25 bp, Artificial sequence
  An exemplary methylation-specific primer (sense)
gtttttgtattttgggagcgcgagc

SEQ ID NO: 59 - DNA, 25 bp, Artificial sequence
  An exemplary methylation-specific primer (sense)
tttgtattttgggagcgcgagcggc

SEQ ID NO: 60 - DNA, 25 bp, Artificial sequence
  An exemplary methylation-specific primer (sense)
tgtattttgggagcgcgagcggcgc

SEQ ID NO: 61 - DNA, 25 bp, Artificial sequence
  An exemplary methylation-specific primer (sense)
tattttgggagcgcgagcggcgcgc

SEQ ID NO: 62 - DNA, 25 bp, Artificial sequence
  An exemplary methylation-specific primer (sense)
ttgggagcgcgagcggcgcgcgggc

SEQ ID NO: 63 - DNA, 25 bp, Artificial sequence
  An exemplary methylation-specific primer (sense)
gcgagcggcgcgcgggcggggaagc

SEQ ID NO: 64 - DNA, 25 bp, Artificial sequence
  An exemplary methylation-specific primer (sense)
gagcggcgcgcgggcggggaagcgc

SEQ ID NO: 65 - DNA, 25 bp, Artificial sequence
  An exemplary methylation-specific primer (sense)
gcggggaagcgcggtttagattttc

SEQ ID NO: 66 - DNA, 25 bp, Artificial sequence
  An exemplary methylation-specific primer (sense)
aagcgcggtttagattttcgggttc

SEQ ID NO: 67 - DNA, 25 bp, Artificial sequence
  An exemplary methylation-specific primer (sense)
gcggtttagattttcgggttcgttc

SEQ ID NO: 68 - DNA, 24 bp, Artificial sequence
  An exemplary methylation-specific primer (sense)
tttgggttcgttcggagtagttgc

SEQ ID NO: 69 - DNA, 25 bp, Artificial sequence
  An exemplary methylation-specific primer (sense)
gttcgttcggagtagttgcgttgtc

SEQ ID NO: 70 - DNA, 25 bp, Artificial sequence
  An exemplary methylation-specific primer (sense)
gtagttgcgttgtcggggttaggtc

SEQ ID NO: 71 - DNA, 25 bp, Artificial sequence
  An exemplary methylation-specific primer (sense)
gttaggtcgggtttttagtggattc

SEQ ID NO: 72 - DNA, 25 bp, Artificial sequence
  An exemplary methylation-specific primer (sense)
taggtcgggtttttagtggattcgc

SEQ ID NO: 73 - DNA, 25 bp, Artificial sequence
  An exemplary methylation-specific primer (sense)
ttttagtggattcgcgggtatagac

SEQ ID NO: 74 - DNA, 25 bp, Artificial sequence
  An exemplary methylation-specific primer (sense)
ttcgcgggtatagacgtttaggatc

SEQ ID NO: 75 - DNA, 25 bp, Artificial sequence
  An exemplary methylation-specific primer (sense)
cgcgggtatagacgtttaggatcgc

SEQ ID NO: 76 - DNA, 25 bp, Artificial sequence
  An exemplary methylation-specific primer (sense)
agacgtttaggatcgcgttttttac

SEQ ID NO: 77 - DNA, 25 bp, Artificial sequence
  An exemplary methylation-specific primer (sense)
tttaggatcgcgttttttacgtggc

SEQ ID NO: 78 - DNA, 25 bp, Artificial sequence
  An exemplary methylation-specific primer (sense)
tacgtggcggagggattggggattc

SEQ ID NO: 79 - DNA, 25 bp, Artificial sequence
  An exemplary methylation-specific primer (sense)
ggagggattggggattcgggtattc

SEQ ID NO: 80 - DNA, 25 bp, Artificial sequence
  An exemplary methylation-specific primer (sense)
tttattttttagtttcgtttttttc

SEQ ID NO: 81 - DNA, 25 bp, Artificial sequence
  An exemplary methylation-specific primer (sense)
tattttttagtttcgtttttttcgc

SEQ ID NO: 82 - DNA, 25 bp, Artificial sequence
  An exemplary methylation-specific primer (sense)
ttttttagtttcgtttttttcgcgc

SEQ ID NO: 83 - DNA, 25 bp, Artificial sequence
  An exemplary methylation-specific primer (sense)
gtttttttcgcgcggattttgtttc

SEQ ID NO: 84 - DNA, 25 bp, Artificial sequence
  An exemplary methylation-specific primer (sense)
tttcgcgcggattttgtttcgtttc

SEQ ID NO: 85 - DNA, 25 bp, Artificial sequence
  An exemplary methylation-specific primer (sense)
attttgtttcgtttcgatttttttc

SEQ ID NO: 86 - DNA, 25 bp, Artificial sequence
  An exemplary methylation-specific primer (sense)
tcgtttcgatttttttcgggttttc

SEQ ID NO: 87 - DNA, 25 bp, Artificial sequence
  An exemplary methylation-specific primer (sense)
tcgggttttcggtttagtttttttc

SEQ ID NO: 88 - DNA, 25 bp, Artificial sequence
  An exemplary methylation-specific primer (sense)
ttttttttttttttttcgcggtttc

SEQ ID NO: 89 - DNA, 25 bp, Artificial sequence
  An exemplary methylation-specific primer (sense)
tttttcgcggtttcgtttttttttc

SEQ ID NO: 90 - DNA, 25 bp, Artificial sequence
  An exemplary methylation-specific primer (sense)
tttcgcggtttcgtttttttttcgc

SEQ ID NO: 91 - DNA, 25 bp, Artificial sequence
  An exemplary methylation-specific primer (anti-sense)
aaacttcccacgtacgcaacaaaac

SEQ ID NO: 92 - DNA, 25 bp, Artificial sequence
  An exemplary methylation-specific primer (anti-sense)
tcccacgtacgcaacaaaacgcaac

SEQ ID NO: 93 - DNA, 25 bp, Artificial sequence
  An exemplary methylation-specific primer (anti-sense)
caaaacgcaacgctacctaaaactc

SEQ ID NO: 94 - DNA, 25 bp, Artificial sequence
  An exemplary methylation-specific primer (anti-sense)
aaacgcaacgctacctaaaactcgc

SEQ ID NO: 95 - DNA, 25 bp, Artificial sequence
  An exemplary methylation-specific primer (anti-sense)
cgcaacgctacctaaaactcgcgcc

SEQ ID NO: 96 - DNA, 25 bp, Artificial sequence
  An exemplary methylation-specific primer (anti-sense)
caacgctacctaaaactcgcgccgc

SEQ ID NO: 97 - DNA, 25 bp, Artificial sequence
  An exemplary methylation-specific primer (anti-sense)
aaaactcgcgccgcgaaaaaaaaac

SEQ ID NO: 98 - DNA, 25 bp, Artificial sequence
  An exemplary methylation-specific primer (anti-sense)
cgcgccgcgaaaaaaaaacgaaacc

SEQ ID NO: 99 - DNA, 25 bp, Artificial sequence
  An exemplary methylation-specific primer (anti-sense)
cgccgcgaaaaaaaaacgaaaccgc

SEQ ID NO: 100 - DNA, 25 bp, Artificial sequence
  An exemplary methylation-specific primer (anti-sense)
aaaaaaacccgaaaaaaactaaacc

SEQ ID NO: 101 - DNA, 25 bp, Artificial sequence
  An exemplary methylation-specific primer (anti-sense)
ccgaaaaaaactaaaccgaaaaccc

SEQ ID NO: 102 - DNA, 25 bp, Artificial sequence
  An exemplary methylation-specific primer (anti-sense)
ctaaaccgaaaacccgaaaaaaatc

SEQ ID NO: 103 - DNA, 25 bp, Artificial sequence
  An exemplary methylation-specific primer (anti-sense)
ccgaaaacccgaaaaaaatcgaaac

SEQ ID NO: 104 - DNA, 25 bp, Artificial sequence
  An exemplary methylation-specific primer (anti-sense)
aaaaaatcgaaacgaaacaaaatcc

SEQ ID NO: 105 - DNA, 25 bp, Artificial sequence
  An exemplary methylation-specific primer (anti-sense)
aaaatcgaaacgaaacaaaatccgc

SEQ ID NO: 106 - DNA, 25 bp, Artificial sequence
  An exemplary methylation-specific primer (anti-sense)
aatcgaaacgaaacaaaatccgcgc

SEQ ID NO: 107 - DNA, 25 bp, Artificial sequence
  An exemplary methylation-specific primer (anti-sense)
gaaacaaaatccgcgcgaaaaaaac

SEQ ID NO: 108 - DNA, 25 bp, Artificial sequence
  An exemplary methylation-specific primer (anti-sense)
aaataaaaaaacaaaacgaataccc

SEQ ID NO: 109 - DNA, 25 bp, Artificial sequence
  An exemplary methylation-specific primer (anti-sense)
gaatacccgaatccccaatccctcc

SEQ ID NO: 110 - DNA, 25 bp, Artificial sequence
  An exemplary methylation-specific primer (anti-sense)
cccgaatccccaatccctccgccac

SEQ ID NO: 111 - DNA, 25 bp, Artificial sequence
  An exemplary methylation-specific primer (anti-sense)
ccaatccctccgccacgtaaaaaac

SEQ ID NO: 112 - DNA, 25 bp, Artificial sequence
  An exemplary methylation-specific primer (anti-sense)
aatccctccgccacgtaaaaaacgc

SEQ ID NO: 113 - DNA, 25 bp, Artificial sequence
  An exemplary methylation-specific primer (anti-sense)
ccacgtaaaaaacgcgatcctaaac

SEQ ID NO: 114 - DNA, 25 bp, Artificial sequence
  An exemplary methylation-specific primer (anti-sense)
aacgcgatcctaaacgtctataccc

SEQ ID NO: 115 - DNA, 25 bp, Artificial sequence
  An exemplary methylation-specific primer (anti-sense)
cgcgatcctaaacgtctatacccgc

SEQ ID NO: 116 - DNA, 25 bp, Artificial sequence
  An exemplary methylation-specific primer (anti-sense)
atacccgcgaatccactaaaaaccc

SEQ ID NO: 117 - DNA, 25 bp, Artificial sequence
  An exemplary methylation-specific primer (anti-sense)
tccactaaaaacccgacctaacccc

SEQ ID NO: 118 - DNA, 25 bp, Artificial sequence
  An exemplary methylation-specific primer (anti-sense)
aaaaacccgacctaaccccgacaac

SEQ ID NO: 119 - DNA, 25 bp, Artificial sequence
  An exemplary methylation-specific primer (anti-sense)
ctaaccccgacaacgcaactactcc

SEQ ID NO: 120 - DNA, 25 bp, Artificial sequence
  An exemplary methylation-specific primer (anti-sense)
ccccgacaacgcaactactccgaac

SEQ ID NO: 121 - DNA, 25 bp, Artificial sequence
  An exemplary methylation-specific primer (anti-sense)
caacgcaactactccgaacgaaccc

SEQ ID NO: 122 - DNA, 25 bp, Artificial sequence
  An exemplary methylation-specific primer (anti-sense)
ccgaacgaacccgaaaatctaaacc

SEQ ID NO: 123 - DNA, 25 bp, Artificial sequence
  An exemplary methylation-specific primer (anti-sense)
gaacgaacccgaaaatctaaaccgc

SEQ ID NO: 124 - DNA, 25 bp, Artificial sequence
  An exemplary methylation-specific primer (anti-sense)
ccgaaaatctaaaccgcgcttcccc

SEQ ID NO: 125 - DNA, 25 bp, Artificial sequence
  An exemplary methylation-specific primer (anti-sense)
aaatctaaaccgcgcttccccgccc

SEQ ID NO: 126 - DNA, 25 bp, Artificial sequence
  An exemplary methylation-specific primer (anti-sense)
atctaaaccgcgcttccccgcccgc

SEQ ID NO: 127 - DNA, 25 bp, Artificial sequence
  An exemplary methylation-specific primer (anti-sense)
ctaaaccgcgcttccccgcccgcgc

SEQ ID NO: 128 - DNA, 25 bp, Artificial sequence
  An exemplary methylation-specific primer (anti-sense)
aaccgcgcttccccgcccgcgcgcc

SEQ ID NO: 129 - DNA, 25 bp, Artificial sequence
  An exemplary methylation-specific primer (anti-sense)
gcgcttccccgcccgcgcgccgctc

SEQ ID NO: 130 - DNA, 25 bp, Artificial sequence
  An exemplary methylation-specific primer (anti-sense)
gcttccccgcccgcgcgccgctcgc

SEQ ID NO: 131 - DNA, 25 bp, Artificial sequence
  An exemplary methylation-specific primer (anti-sense)
gctcgcgctcccaaaatacaaaaac

SEQ ID NO: 132 - DNA, 25 bp, Artificial sequence
  An exemplary methylation-specific primer (anti-sense)
gctcccaaaatacaaaaacgccaac

SEQ ID NO: 133 - DNA, 25 bp, Artificial sequence
  An exemplary methylation-specific primer (anti-sense)
caaaaacgccaacgaaaaccccaac

SEQ ID NO: 134 - DNA, 25 bp, Artificial sequence
  An exemplary methylation-specific primer (anti-sense)
acgaaaaccccaacgaaaaaaaatc

SEQ ID NO: 135 - DNA, 25 bp, Artificial sequence
  An exemplary methylation-specific primer (anti-sense)
aaccccaacgaaaaaaaatcgaatc

SEQ ID NO: 136 - DNA, 25 bp, Artificial sequence
  An exemplary methylation-specific primer (anti-sense)
atcgacctaaactataaaataaccc

SEQ ID NO: 137 - DNA, 25 bp, Artificial sequence
  An exemplary methylation-specific primer (anti-sense)
aaaaaccctaaaaacaaatacgtac

SEQ ID NO: 138 - DNA, 25 bp, Artificial sequence
  An exemplary methylation-specific primer (anti-sense)
aaccctaaaaacaaatacgtacgac

SEQ ID NO: 139 - DNA, 25 bp, Artificial sequence
  An exemplary methylation-specific primer (anti-sense)
aaatacgtacgacgaccctttaacc

SEQ ID NO: 140 - DNA, 25 bp, Artificial sequence
  An exemplary methylation-specific primer (anti-sense)
gaccctttaaccgctaacctaatcc

SEQ ID NO: 141 - DNA, 25 bp, Artificial sequence
  An exemplary methylation-specific primer (anti-sense)
cccaaaactacctccaaatccgaac

SEQ ID NO: 142 - DNA, 25 bp, Artificial sequence
  An exemplary methylation-specific primer (anti-sense)
caaaactacctccaaatccgaacgc

SEQ ID NO: 143 - DNA, 25 bp, Artificial sequence
  An exemplary methylation-specific primer (anti-sense)
ctacctccaaatccgaacgcgaaac

SEQ ID NO: 144 - DNA, 25 bp, Artificial sequence
  An exemplary methylation-specific primer (anti-sense)
cctccaaatccgaacgcgaaacgtc

SEQ ID NO: 145 - DNA, 25 bp, Artificial sequence
  An exemplary methylation-specific primer (anti-sense)
atccgaacgcgaaacgtcgaactcc

SEQ ID NO: 146 - DNA, 25 bp, Artificial sequence
  An exemplary methylation-specific primer (anti-sense)
cgaaacgtcgaactccgaacaccac

SEQ ID NO: 147 - DNA, 25 bp, Artificial sequence
  An exemplary methylation-specific primer (anti-sense)
tcgaactccgaacaccacgaatacc

SEQ ID NO: 148 - DNA, 25 bp, Artificial sequence
  An exemplary methylation-specific primer (anti-sense)
actccgaacaccacgaataccgaac

SEQ ID NO: 149 - DNA, 25 bp, Artificial sequence
  An exemplary methylation-specific primer (anti-sense)
gaataccgaacgtaaaaaaaaaaac

SEQ ID NO: 150 - DNA, 25 bp, Artificial sequence
  An exemplary methylation-specific primer (anti-sense)
cgaacgtaaaaaaaaaaacgaaaac

SEQ ID NO: 151 - DNA, 25 bp, Artificial sequence
  An exemplary methylation-specific primer (anti-sense)
aacgtaaaaaaaaaaacgaaaacgc

SEQ ID NO: 152 - DNA, 25 bp, Artificial sequence
  An exemplary methylation-specific primer (anti-sense)
aaaaaaaaaacgaaaacgcgtaaac

SEQ ID NO: 153 - DNA, 25 bp, Artificial sequence
  An exemplary methylation-specific primer (anti-sense)
aaaaaaaacgaaaacgcgtaaacgc

SEQ ID NO: 154 - DNA, 25 bp, Artificial sequence
  An exemplary methylation-specific primer (anti-sense)
aaaacgcgtaaacgcgactaaaaac

SEQ ID NO: 155 - DNA, 25 bp, Artificial sequence
  An exemplary methylation-specific primer (anti-sense)
cgtaaacgcgactaaaaacgaaccc

SEQ ID NO: 156 - DNA, 25 bp, Artificial sequence
  An exemplary methylation-specific primer (anti-sense)
cgcgactaaaaacgaacccgaaaac

SEQ ID NO: 157 - DNA, 25 bp, Artificial sequence
  An exemplary methylation-specific primer (anti-sense)
cccgaaaacgcattactccctaaac

SEQ ID NO: 158 - DNA, 25 bp, Artificial sequence
  An exemplary methylation-specific primer (anti-sense)
aacgcattactccctaaacgaacac

SEQ ID NO: 159 - DNA, 25 bp, Artificial sequence
  An exemplary methylation-specific primer (anti-sense)
cgcattactccctaaacgaacacgc

SEQ ID NO: 160 - DNA, 25 bp, Artificial sequence
  An exemplary methylation-specific primer (anti-sense)
cctaaacgaacacgcgaaacctccc

SEQ ID NO: 161 - DNA, 25 bp, Artificial sequence
  An exemplary methylation-specific primer (anti-sense)
atacctccctacaacacttccccgc

SEQ ID NO: 162 - DNA, 25 bp, Artificial sequence
  An exemplary methylation-specific primer (anti-sense)
gacttaaactccttaacacaaaccc

SEQ ID NO: 163 - DNA, 25 bp, Artificial sequence
  An exemplary methylation-specific primer (anti-sense)
ttctctttacaaattctcaaacgac

SEQ ID NO: 164 - DNA, 25 bp, Artificial sequence
  An exemplary methylation-specific primer (anti-sense)
aaatctattaatcacccaccgaaac

SEQ ID NO: 165 - DNA, 25 bp, Artificial sequence
  An exemplary methylation-specific primer (anti-sense)
attaatcacccaccgaaacgatccc

SEQ ID NO: 166 - DNA, 25 bp, Artificial sequence
  An exemplary methylation-specific primer (anti-sense)
aatcacccaccgaaacgatcccgtc

SEQ ID NO: 167 - DNA, 25 bp, Artificial sequence
  An exemplary methylation-specific primer (anti-sense)
ataaaaccaaacgctcctactaacc

SEQ ID NO: 168 - DNA, 25 bp, Artificial sequence
  An exemplary methylation-specific primer (anti-sense)
aaaaccaaacgctcctactaaccgc

SEQ ID NO: 169 - DNA, 25 bp, Artificial sequence
  An exemplary methylation-specific primer (anti-sense)
caaacgctcctactaaccgcgcacc

SEQ ID NO: 170 - DNA, 25 bp, Artificial sequence
  An exemplary methylation-specific primer (anti-sense)
cgctcctactaaccgcgcaccgaac

SEQ ID NO: 171 - DNA, 25 bp, Artificial sequence
  An exemplary methylation-specific primer (anti-sense)
ccgaacgcctcacaccaaccacaac

SEQ ID NO: 172 - DNA, 25 bp, Artificial sequence
  An exemplary methylation-specific primer (anti-sense)
cacaacgaccttaaccctaaacccc

SEQ ID NO: 173 - DNA, 25 bp, Artificial sequence
  An exemplary methylation-specific primer (anti-sense)
accaacatctaatcacatcccgccc

SEQ ID NO: 174 - DNA, 25 bp, Artificial sequence
  An exemplary methylation-specific primer (anti-sense)
cccgcacaaaataaaaaacaacctc

SEQ ID NO: 175 - DNA, 21 bp, Artificial sequence
  Cloning primer - outer sense
gggtttgtgttaaggagttta

SEQ ID NO: 176 - DNA, 21 bp, Artificial sequence
  Cloning primer - outer antisense
accataatataaaaaccctaa

SEQ ID NO: 177 - DNA, 23 bp, Artificial sequence
  Cloning primer - inner sense
ggtttgtgttaaggagtttaagt

SEQ ID NO: 178 - DNA, 25 bp, Artificial sequence
  Cloning primer - inner antisense
atataaaaaccctaaaaacaaatac

SEQ ID NO: 179 - DNA, 21 bp, Artificial sequence
  Exemplary methylation-specific primer - sense
ttcgggaggtttcgcgtgttc

SEQ ID NO: 180 - DNA, 21 bp, Artificial sequence
  Exemplary methylation-specific primer - antisense
tccaaatccgaacgcgaaacg

SEQ ID NO: 181 - DNA, 22 bp, Artificial sequence
  Exemplary normalization primer - sense
gatttggggtggtttgtttatg

SEQ ID NO: 182 - DNA, 23 bp, Artificial sequence
  Exemplary normalization primer - antisense
aatacctccctacaacacttccc